European Patent Specification EP 4 039 812 B1, published June 11, 2025. Title: REGENERATING FUNCTIONAL NEURONS FOR TREATMENT OF NEURAL INJURY CAUSED BY DISRUPTION OF BLOOD FLOW. Applicant: The Penn State Research Foundation. The sequence listing filed with the application follows.

SEQUENCE LISTING (9 sequences)

SEQ ID NO: 1 - DNA, 1071 bp, Homo sapiens
atgaccaaatcgtacagcgagagtgggctgatgggcgagcctcagccccaaggtcctccaagctggacagacgagtgtctcagttctcaggacgaggagcacgaggcagacaagaaggaggacgacctcgaagccatgaacgcagaggaggactcactgaggaacgggggagaggaggaggacgaagatgaggacctggaagaggaggaagaagaggaagaggaggatgacgatcaaaagcccaagagacgcggccccaaaaagaagaagatgactaaggctcgcctggagcgttttaaattgagacgcatgaaggctaacgcccgggagcggaaccgcatgcacggactgaacgcggcgctagacaacctgcgcaaggtggtgccttgctattctaagacgcagaagctgtccaaaatcgagactctgcgcttggccaagaactacatctgggctctgtcggagatcctgcgctcaggcaaaagcccagacctggtctccttcgttcagacgctttgcaagggcttatcccaacccaccaccaacctggttgcgggctgcctgcaactcaatcctcggacttttctgcctgagcagaaccaggacatgcccccccacctgccgacggccagcgcttccttccctgtacacccctactcctaccagtcgcctgggctgcccagtccgccttacggtaccatggacagctcccatgtcttccacgttaagcctccgccgcacgcctacagcgcagcgctggagcccttctttgaaagccctctgactgattgcaccagcccttcctttgatggacccctcagcccgccgctcagcatcaatggcaacttctctttcaaacacgaaccgtccgccgagtttgagaaaaattatgcctttaccatgcactatcctgcagcgacactggcaggggcccaaagccacggatcaatcttctcaggcaccgctgcccctcgctgcgagatccccatagacaatattatgtccttcgatagccattcacatcatgagcgagtcatgagtgcccagctcaatgccatatttcatgattag

SEQ ID NO: 2 - protein, 356 aa, Homo sapiens
MTKSYSESGLMGEPQPQGPPSWTDECLSSQDEEHEADKKEDDLEAMNAEEDSLRNGGEEEDEDEDLEEEEEEEEEDDDQKPKRRGPKKKKMTKARLERFKLRRMKANARERNRMHGLNAALDNLRKVVPCYSKTQKLSKIETLRLAKNYIWALSEILRSGKSPDLVSFVQTLCKGLSQPTTNLVAGCLQLNPRTFLPEQNQDMPPHLPTASASFPVHPYSYQSPGLPSPPYGTMDSSHVFHVKPPPHAYSAALEPFFESPLTDCTSPSFDGPLSPPLSINGNFSFKHEPSAEFEKNYAFTMHYPAATLAGAQSHGSIFSGTAAPRCEIPIDNIMSFDSHSHHERVMSAQLNAIFHD

SEQ ID NO: 3 - DNA, 1074 bp, Mus musculus
atgaccaaatcatacagcgagagcgggctgatgggcgagcctcagccccaaggtcccccaagctggacagatgagtgtctcagttctcaggacgaggaacacgaggcagacaagaaagaggacgagcttgaagccatgaatgcagaggaggactctctgagaaacgggggagaggaggaggaggaagatgaggatctagaggaagaggaggaagaagaagaggaggaggaggatcaaaagcccaagagacggggtcccaaaaagaaaaagatgaccaaggcgcgcctagaacgttttaaattaaggcgcatgaaggccaacgcccgcgagcggaaccgcatgcacgggctgaacgcggcgctggacaacctgcgcaaggtggtaccttgctactccaagacccagaaactgtctaaaatagagacactgcgcttggccaagaactacatctgggctctgtcagagatcctgcgctcaggcaaaagccctgatctggtctccttcgtacagacgctctgcaaaggtttgtcccagcccactaccaatttggtcgccggctgcctgcagctcaaccctcggactttcttgcctgagcagaacccggacatgcccccgcatctgccaaccgccagcgcttccttcccggtgcatccctactcctaccagtcccctggactgcccagcccgccctacggcaccatggacagctcccacgtcttccacgtcaagccgccgccacacgcctacagcgcagctctggagcccttctttgaaagccccctaactgactgcaccagcccttcctttgacggacccctcagcccgccgctcagcatcaatggcaacttctctttcaaacacgaaccatccgccgagtttgaaaaaaattatgcctttaccatgcactaccctgcagcgacgctggcagggccccaaagccacggatcaatcttctcttccggtgccgctgcccctcgctgcgagatccccatagacaacattatgtctttcgatagccattcgcatcatgagcgagtcatgagtgcccagcttaatgccatctttcacgattag

SEQ ID NO: 4 - protein, 357 aa, Mus musculus
MTKSYSESGLMGEPQPQGPPSWTDECLSSQDEEHEADKKEDELEAMNAEEDSLRNGGEEEEEDEDLEEEEEEEEEEEDQKPKRRGPKKKKMTKARLERFKLRRMKANARERNRMHGLNAALDNLRKVVPCYSKTQKLSKIETLRLAKNYIWALSEILRSGKSPDLVSFVQTLCKGLSQPTTNLVAGCLQLNPRTFLPEQNPDMPPHLPTASASFPVHPYSYQSPGLPSPPYGTMDSSHVFHVKPPPHAYSAALEPFFESPLTDCTSPSFDGPLSPPLSINGNFSFKHEPSAEFEKNYAFTMHYPAATLAGPQSHGSIFSSGAAAPRCEIPIDNIMSFDSHSHHERVMSAQLNAIFHD

SEQ ID NO: 5 - DNA, 1053 bp, Mus musculus
gcagtgtggagacacacccactttccccaagggctcctgctcccccaagtgatccccttatcctccgtgctaagatgacaccgaggttgcagtccttacctttgaaagcagccacaagggcgtgggggtgcacacctttaatcccagcactcgggaggcagaggcaggcagatttctgagttcgagaccagcctggtctacaaagtgaattccaggacagccagggctatacagagaaaccctgtcttgaaaaaaaaagagaaagaaaaaagaaaaaaaaaaatgaaagcagccacatctaaggactacgtggcacaggagagggtgagtccctgagagttcagctgctgccctgtctgttcctgtaaatggcagtggggtcatgggaaagtgaaggggctcaaggtattggacacttccaggataatcttttggacgcctcaccctgtgccaggaccaaggctgagcttggcaggctcagaacagggtgtcctgttcttccctgtctaaaacattcactctcagcttgctcacccttccccagacaaggaagctgcacagggtctggtgttcagatggctttggcttacagcaggtgtgggtgtggggtaggaggcagggggtaggggtgggggaagcctgtactatactcactatcctgtttctgaccctctaggactcctacagggttatgggagtggacaggcagtccagatctgagctgctgacccacaagcagtgccctgtgcctgccagaatccaaagccctgggaatgtccctctggtccccctctgtcccctgcagcccttcctgttgctcaaccttgcacagttccgacctgggggagagagggacagaaatcttgccaagtatttcaacagaatgtactggcaattacttcatggcttcctggacttggtaaaggatggactaccccgcccaacaggggggctggcagccaggtaggcccataaaaagcccgctggggagtcctcctcactctctgctcttcctcctccagcacacatcagacctagtagctgtggaaacca

SEQ ID NO: 6 - DNA, 1672 bp, Homo sapiens
gtctgcaagcagacctggcagcattgggctggccgccccccagggcctcctcttcatgcccagtgaatgactcaccttggcacagacacaatgttcggggtgggcacagtgcctgcttcccgccgcaccccagcccccctcaaatgccttccgagaagcccattgagtagggggcttgcattgcaccccagcctgacagcctggcatcttgggataaaagcagcacagccccctaggggctgcccttgctgtgtggcgccaccggcggtggagaacaaggctctattcagcctgtgcccaggaaaggggatcaggggatgcccaggcatggacagtgggtggcagggggggagaggagggctgtctgcttcccagaagtccaaggacacaaatgggtgaggggactgggcagggttctgaccctgtgggaccagagtggagggcgtagatggacctgaagtctccagggacaacagggcccaggtctcaggctcctagttgggcccagtggctccagcgtttccaaacccatccatccccagaggttcttcccatctctccaggctgatgtgtgggaactcgaggaaataaatctccagtgggagacggaggggtggccagggaaacggggcgctgcaggaataaagacgagccagcacagccagctcatgcgtaacggctttgtggagctgtcaaggcctggtctctgggagagaggcacagggaggccagacaaggaaggggtgacctggagggacagatccaggggctaaagtcctgataaggcaagagagtgccggccccctcttgccctatcaggacctccactgccacatagaggccatgattgacccttagacaaagggctggtgtccaatcccagcccccagccccagaactccagggaatgaatgggcagagagcaggaatgtgggacatctgtgttcaagggaaggactccaggagtctgctgggaatgaggcctagtaggaaatgaggtggcccttgagggtacagaacaggttcattcttcgccaaattcccagcaccttgcaggcacttacagctgagtgagataatgcctgggttatgaaatcaaaaagttggaaagcaggtcagaggtcatctggtacagcccttccttccctttttttttttttttttttgtgagacaaggtctctctctgttgcccaggctggagtggcgcaaacacagctcactgcagcctcaacctactgggctcaagcaatcctccagcctcagcctcccaaagtgctgggattacaagcatgagccaccccactcagccctttccttcctttttaattgatgcataataattgtaagtattcatcatggtccaaccaaccctttcttgacccaccttcctagagagagggtcctcttgattcagcggtcagggccccagacccatggtctggctccaggtaccacctgcctcatgcaggagttggcgtgcccaggaagctctgcctctgggcacagtgacctcagtggggtgaggggagctctccccatagctgggctgcggcccaaccccaccccctcaggctatgccagggggtgttgccaggggcacccgggcatcgccagtctagcccactccttcataaagccctcgcatcccaggagcgagcagagccagagcat

SEQ ID NO: 7 - DNA, 1610 bp, Mus musculus
aactgagagtggaggggcacagaagagcccaagaggctccttaggttgtgtggagggtacaatatgtttgggctgagcaacccagagccagactttgtctggctggtaagagacagaggtgcctgctatcacaatccaagggtctgcttgaggcagagccagtgcaaaggatgtggttagagccagcctggtgtactgaagaggggcgaagagcttgagtaaggagtctcagcggtggtttgagaggcagggtggttaatggagtagctgcaggggagaatccttgggagggagcctgcaggacagagctttggtcaggaagtgatgggcatgtcactggaccctgtattgtctctgacttttctcaagtaggacaatgactctgcccagggagggggtctgtgacaaggtggaagggccagaggagaacttctgagaagaaaaccagaggccgtgaagaggtgggaagggcatgggattcagaacctcaggcccaccaggacacaaccccaggtccacagcagatgggtgaccttgcatgtctcagtcaccagcattgtgctccttgcttatcacgcttgggtgaaggaaatgacccaaatagcataaagcctgaaggccgggactaggccagctagggcttgcccttcccttcccagctgcactttccataggtcccaccttcagcagattagacccgcctcctgcttcctgcctccttgcctcctcactcatgggtctatgcccacctccagtctcgggactgaggctcactgaagtcccatcgaggtctggtctggtgaatcagcggctggctctgggccctgggcgaccagttaggttccgggcatgctaggcaatgaactctacccggaattgggggtgcggggaggcggggaggtctccaacccagccttttgaggacgtgcctgtcgctgcacggtgctttttatagacgatggtggcccattttgcagaagggaaagccggagccctctggggagcaaggtccccgcaaatggacggatgacctgagcttggttctgccagtccacttcccaaatccctcaccccattctagggactagggaaagatctcctgattggtcatatctgggggcctggccggagggcctcctatgattggagagatctaggctgggcgggccctagagcccgcctcttctctgcctggaggaggagcactgaccctaaccctctctgcacaagacccgagcttgtgcgcccttctgggagcttgctgcccctgtgctgactgctgacagctgactgacgctcgcagctagcaggtacttctgggttgctagcccagagccctgggccggtgaccctgttttccctacttcccgtctttgaccttgggtaagtttctttttcttttgtttttgagagaggcacccagatcctctccactacaggcagccgctgaaccttggatcctcagctcctgccctgggaactacagttcctgccctttttttcccaccttgagggaggttttccctgagtagcttcgactatcctggaacaagctttgtagaccagcctgggtctccggagagttgggattaaaggcgtgcaccaccacc

SEQ ID NO: 8 - DNA, 1387 bp, Homo sapiens
ctctggtttcaagaccaatactcataacccccacatggaccaggcaccatcacacctgagcactgcacttagggtcaaagacctggccccacatctcagcagctatgtagactagctccagtcccttaatctctctcagcctcagtttcttcatctgcaaaacaggtctcagtttcgttgcaaagtatgaagtgctgggctgttactggtcaaagggaagagctgggaagagggtgcaaggtggggttgggctggagatgggctggagcagatagatggagggacctgaatggaggaagtaaaccaaggcccggtaacattgggactggacagagaacacgcagatcctctaggcaccggaagctaagtaacattgccctttctcctcctgtttgggactaggctgatgttgctgcctggaagggagccagcagaagggccccagcctgaagctgttaggtagaagccaaatccagggccagatttccaggaggcagcctcgggaagttgaaacacccggattcaggggtcaggaggcctgggcttctggcaccaaacggccagggacctactttccacctggagtcttgtaagagccactttcagcttgagctgcactttcgtcctccatgaaatgggggaggggatgctcctcacccaccttgcaaggttattttgaggcaaatgtcatggcgggactgagaattcttctgccctgcgaggaaatccagacatctctcccttacagacagggagactgaggtgaggcccttccaggcagagaaggtcactgttgcagccatgggcagtgccccacaggacctcgggtggtgcctctggagtctggagaagttcctaggggacctccgaggcaaagcagcccaaaagccgcctgtgagggtggctggtgtctgtccttcctcctaaggctggagtgtgcctgtggaggggtctcctgaactcccgcaaaggcagaaaggagggaagtaggggctgggacagttcatgcctcctccctgagggggtctcccgggctcggctcttggggccagagttcagggtgtctgggcctctctatgactttgttctaagtctttagggtggggctggggtctggcccagctgcaagggccccctcacccctgccccagagaggaacagccccgcacgggccctttaagaaggttgagggtgggggcaggtgggggagtccaagcctgaaacccgagcgggcgcgcgggtctgcgcctgccccgcccccggagttaagtgcgcggacacccggagccggcccgcgcccaggagcagagccgcgctcgctccactcagctcccagctcccaggactccgctggctcctcgcaagtcctgccgcccagcccgccggg

SEQ ID NO: 9 - DNA, 9232 bp, Artificial Sequence
  Construct including CAG promoter and encoding NeuroD1 and green fluoresecent protein separated by an IRES.
gatccggccattagccatattattcattggttatatagcataaatcaatattggctattggccattgcatacgttgtatccatatcataatatgtacatttatattggctcatgtccaacattaccgccatgttgacattgattattgactagttattaatagtaatcaattacggggtcattagttcatagcccatatatggagttccgcgttacataacttacggtaaatggcccgcctggctgaccgcccaacgacccccgcccattgacgtcaataatgacgtatgttcccatagtaacgccaatagggactttccattgacgtcaatgggtggagtatttacggtaaactgcccacttggcagtacatcaagtgtatcatatgccaagtacgccccctattgacgtcaatgacggtaaatggcccgcctggcattatgcccagtacatgaccttatgggactttcctacttggcagtacatctacgtattagtcatcgctattaccatggtgatgcggttttggcagtacatcaatgggcgtggatagcggtttgactcacggggatttccaagtctccaccccattgacgtcaatgggagtttgttttggcaccaaaatcaacgggactttccaaaatgtcgtaacaactccgccccattgacgcaaatgggcggtaggcatgtacggtgggaggtctatataagcagagctcaataaaagagcccacaacccctcactcggggcgccagtcctccgattgactgagtcgcccgggtacccgtattcccaataaagcctcttgctgtttgcatccgaatcgtggtctcgctgttccttgggagggtctcctctgagtgattgactacccacgacgggggtctttcatttgggggctcgtccgggatttggagacccctgcccagggaccaccgacccaccaccgggaggtaagctggccagcaacttatctgtgtctgtccgattgtctagtgtctatgtttgatgttatgcgcctgcgtctgtactagttagctaactagctctgtatctggcggacccgtggtggaactgacgagttctgaacacccggccgcaaccctgggagacgtcccagggactttgggggccgtttttgtggcccgacctgaggaagggagtcgatgtggaatccgaccccgtcaggatatgtggttctggtaggagacgagaacctaaaacagttcccgcctccgtctgaatttttgctttcggtttggaaccgaagccgcgcgtcttgtctgctgcagcgctgcagcatcgttctgtgttgtctctgtctgactgtgtttctgtatttgtctgaaaattagggccagactgttaccactcccttaagtttgaccttaggtcactggaaagatgtcgagcggatcgctcacaaccagtcggtagatgtcaagaagagacgttgggttaccttctgctctgcagaatggccaacctttaacgtcggatggccgcgagacggcacctttaaccgagacctcatcacccaggttaagatcaaggtcttttcacctggcccgcatggacacccagaccaggtcccctacatcgtgacctgggaagccttggcttttgacccccctccctgggtcaagccctttgtacaccctaagcctccgcctcctcttcctccatccgccccgtctctcccccttgaacctcctcgttcgaccccgcctcgatcctccctttatccagccctcactccttctctaggcgccggaattcgatgtcgacattgattattgactagttattaatagtaatcaattacggggtcattagttcatagcccatatatggagttccgcgttacataacttacggtaaatggcccgcctggctgaccgcccaacgacccccgcccattgacgtcaataatgacgtatgttcccatagtaacgccaatagggactttccattgacgtcaatgggtggactatttacggtaaactgcccacttggcagtacatcaagtgtatcatatgccaagtacgccccctattgacgtcaatgacggtaaatggcccgcctggcattatgcccagtacatgaccttatgggactttcctacttggcagtacatctacgtattagtcatcgctattaccatgggtcgaggtgagccccacgttctgcttcactctccccatctcccccccctccccacccccaattttgtatttatttattttttaattattttgtgcagcgatgggggcggggggggggggggcgcgcgccaggcggggcggggcggggcgaggggcggggcggggcgaggcggagaggtgcggcggcagccaatcagagcggcgcgctccgaaagtttccttttatggcgaggcggcggcggcggcggccctataaaaagcgaagcgcgcggcgggcgggagtcgctgcgttgccttcgccccgtgccccgctccgcgccgcctcgcgccgcccgccccggctctgactgaccgcgttactcccacaggtgagcgggcgggacggcccttctcctccgggctgtaattagcgcttggtttaatgacggctcgtttcttttctgtggctgcgtgaaagccttaaagggctccgggagggccctttgtgcgggggggagcggctcggggggtgcgtgcgtgtgtgtgtgcgtggggagcgccgcgtgcggcccgcgctgcccggcggctgtgagcgctgcgggcgcggcgcggggctttgtgcgctccgcgtgtgcgcgaggggagcgcggccgggggcggtgccccgcggtgcgggggggctgcgaggggaacaaaggctgcgtgcggggtgtgtgcgtgggggggtgagcagggggtgtgggcgcggcggtcgggctgtaacccccccctgcacccccctccccgagttgctgagcacggcccggcttcgggtgcggggctccgtgcggggcgtggcgcggggctcgccgtgccgggcggggggtggcggcaggtgggggtgccgggcggggcggggccgcctcgggccggggagggctcgggggaggggcgcggcggccccggagcgccggcggctgtcgaggcgcggcgagccgcagccattgccttttatggtaatcgtgcgagagggcgcagggacttcctttgtcccaaatctggcggagccgaaatctgggaggcgccgccgcaccccctctagcgggcgcgggcgaagcggtgcggcgccggcaggaaggaaatgggcggggagggccttcgtgcgtcgccgcgccgccgtccccttctccatctccagcctcggggctgccgcagggggacggctgccttcgggggggacggggcagggcggggttcggcttctggcgtgtgaccggcggctctagagcctctgctaaccatgttcatgccttcttctttttcctacagctcctgggcaacgtgctggttgttgtgctgtctcatcattttggcaaagaattcgctagcggatccggccgcctcggccaccggtcgccaccatcgccaccatgaccaaatcatacagcgagagcgggctgatgggcgagcctcagccccaaggtcccccaagctggacagatgagtgtctcagttctcaggacgaggaacacgaggcagacaagaaagaggacgagcttgaagccatgaatgcagaggaggactctctgagaaacgggggagaggaggaggaggaagatgaggatctagaggaagaggaggaagaagaagaggaggaggaggatcaaaagcccaagagacggggtcccaaaaagaaaaagatgaccaaggcgcgcctagaacgttttaaattaaggcgcatgaaggccaacgcccgcgagcggaaccgcatgcacgggctgaacgcggcgctggacaacctgcgcaaggtggtaccttgctactccaagacccagaaactgtctaaaatagagacactgcgcttggccaagaactacatctgggctctgtcagagatcctgcgctcaggcaaaagccctgatctggtctccttcgtacagacgctctgcaaaggtttgtcccagcccactaccaatttggtcgccggctgcctgcagctcaaccctcggactttcttgcctgagcagaacccggacatgcccccgcatctgccaaccgccagcgcttccttcccggtgcatccctactcctaccagtcccctggactgcccagcccgccctacggcaccatggacagctcccacgtcttccacgtcaagccgccgccacacgcctacagcgcagctctggagcccttctttgaaagccccctaactgactgcaccagcccttcctttgacggacccctcagcccgccgctcagcatcaatggcaacttctctttcaaacacgaaccatccgccgagtttgaaaaaaattatgcctttaccatgcactaccctgcagcgacgctggcagggccccaaagccacggatcaatcttctcttccggtgccgctgcccctcgctgcgagatccccatagacaacattatgtctttcgatagccattcgcatcatgagcgagtcatgagtgcccagcttaatgccatctttcacgattaggtttaaacgcggccgcgcccctctccctcccccccccctaacgttactggccgaagccgcttggaataaggccggtgtgcgtttgtctatatgttattttccaccatattgccgtcttttggcaatgtgagggcccggaaacctggccctgtcttcttgacgagcattcctaggggtctttcccctctcgccaaaggaatgcaaggtctgttgaatgtcgtgaaggaagcagttcctctggaagcttcttgaagacaaacaacgtctgtagcgaccctttgcaggcagcggaaccccccacctggcgacaggtgcctctgcggccaaaagccacgtgtataagatacacctgcaaaggcggcacaaccccagtgccacgttgtgagttggatagttgtggaaagagtcaaatggctctcctcaagcgtattcaacaaggggctgaaggatgcccagaaggtaccccattgtatgggatctgatctggggcctcggtgcacatgctttacatgtgtttagtcgaggttaaaaaaacgtctaggccccccgaaccacggggacgtggttttcctttgaaaaacacgatgataatatggccacaaccatggtgagcaagggcgaggagctgttcaccggggtggtgcccatcctggtcgagctggacggcgacgtaaacggccacaagttcagcgtgtccggcgagggcgagggcgatgccacctacggcaagctgaccctgaagttcatctgcaccaccggcaagctgcccgtgccctggcccaccctcgtgaccaccctgacctacggcgtgcagtgcttcagccgctaccccgaccacatgaagcagcacgacttcttcaagtccgccatgcccgaaggctacgtccaggagcgcaccatcttcttcaaggacgacggcaactacaagacccgcgccgaggtgaagttcgagggcgacaccctggtgaaccgcatcgagctgaagggcatcgacttcaaggaggacggcaacatcctggggcacaagctggagtacaactacaacagccacaacgtctatatcatggccgacaagcagaagaacggcatcaaggtgaacttcaagatccgccacaacatcgaggacggcagcgtgcagctcgccgaccactaccagcagaacacccccatcggcgacggccccgtgctgctgcccgacaaccactacctgagcacccagtccgccctgagcaaagaccccaacgagaagcgcgatcacatggtcctgctggagttcgtgaccgccgccgggatcactctcggcatggacgagctgtacaagtaagtcgacaatcaacctctggattacaaaatttgtgaaagattgactggtattcttaactatgttgctccttttacgctatgtggatacgctgctttaatgcctttgtatcatgctattgcttcccgtatggctttcattttctcctccttgtataaatcctggttgctgtctctttatgaggagttgtggcccgttgtcaggcaacgtggcgtggtgtgcactgtgtttgctgacgcaacccccactggttggggcattgccaccacctgtcagctcctttccgggactttcgctttccccctccctattgccacggcggaactcatcgccgcctgccttgcccgctgctggacaggggctcggctgttgggcactgacaattccgtggtgttgtcggggaagctgacgtcctttccatggctgctcgcctgtgttgccacctggattctgcgcgggacgtccttctgctacgtcccttcggccctcaatccagcggaccttccttcccgcggcctgctgccggctctgcggcctcttccgcgtcttcgccttcgccctcagacgagtcggatctccctttgggccgcctccccgcctggaattcgagctcgagcttgttaacatcgataaaataaaagattttatttagtctccagaaaaaggggggaatgaaagaccccacctgtaggtttggcaagctagcttaagtaacgccattttgcaaggcatggaaaaatacataactgagaatagagaagttcagatcaaggtcaggaacagatggaacagctgaatatgggccaaacaggatatctgtggtaagcagttcctgccccggctcagggccaagaacagatggaacagctgaatatgggccaaacaggatatctgtggtaagcagttcctgccccggctcagggccaagaacagatggtccccagatgcggtccagccctcagcagtttctagagaaccatcagatgtttccagggtgccccaaggacctgaaatgaccctgtgccttatttgaactaaccaatcagttcgcttctcgcttctgttcgcgcgcttctgctccccgagctcaataaaagagcccacaacccctcactcggggcgccagtcctccgattgactgagtcgcccgggtacccgtgtatccaataaaccctcttgcagttgcatccgacttgtggtctcgctgttccttgggagggtctcctctgagtgattgactacccgtcagcgggggtctttcatttccgacttgtggtctcgctgccttgggagggtctcctctgagtgattgactacccgtcagcgggggtcttcacatgcagcatgtatcaaaattaatttggttttttttcttaagtatttacattaaatggccatagttgcattaatgaatcggccaacgcgcggggagaggcggtttgcgtattggcgctcttccgcttcctcgctcactgactcgctgcgctcggtcgttcggctgcggcgagcggtatcagctcactcaaaggcggtaatacggttatccacagaatcaggggataacgcaggaaagaacatgtgagcaaaaggccagcaaaaggccaggaaccgtaaaaaggccgcgttgctggcgtttttccataggctccgcccccctgacgagcatcacaaaaatcgacgctcaagtcagaggtggcgaaacccgacaggactataaagataccaggcgtttccccctggaagctccctcgtgcgctctcctgttccgaccctgccgcttaccggatacctgtccgcctttctcccttcgggaagcgtggcgctttctcatagctcacgctgtaggtatctcagttcggtgtaggtcgttcgctccaagctgggctgtgtgcacgaaccccccgttcagcccgaccgctgcgccttatccggtaactatcgtcttgagtccaacccggtaagacacgacttatcgccactggcagcagccactggtaacaggattagcagagcgaggtatgtaggcggtgctacagagttcttgaagtggtggcctaactacggctacactagaaggacagtatttggtatctgcgctctgctgaagccagttaccttcggaaaaagagttggtagctcttgatccggcaaacaaaccaccgctggtagcggtggtttttttgtttgcaagcagcagattacgcgcagaaaaaaaggatctcaagaagatcctttgatcttttctacggggtctgacgctcagtggaacgaaaactcacgttaagggattttggtcatgagattatcaaaaaggatcttcacctagatccttttaaattaaaaatgaagtttgcggccggccgcaaatcaatctaaagtatatatgagtaaacttggtctgacagttaccaatgcttaatcagtgaggcacctatctcagcgatctgtctatttcgttcatccatagttgcctgactccccgtcgtgtagataactacgatacgggagggcttaccatctggccccagtgctgcaatgataccgcgagacccacgctcaccggctccagatttatcagcaataaaccagccagccggaagggccgagcgcagaagtggtcctgcaactttatccgcctccatccagtctattaattgttgccgggaagctagagtaagtagttcgccagttaatagtttgcgcaacgttgttgccattgctacaggcatcgtggtgtcacgctcgtcgtttggtatggcttcattcagctccggttcccaacgatcaaggcgagttacatgatcccccatgttgtgcaaaaaagcggttagctccttcggtcctccgatcgttgtcagaagtaagttggccgcagtgttatcactcatggttatggcagcactgcataattctcttactgtcatgccatccgtaagatgcttttctgtgactggtgagtactcaaccaagtcattctgagaatagtgtatgcggcgaccgagttgctcttgcccggcgtcaacacgggataataccgcgccacatagcagaactttaaaagtgctcatcattggaaaacgttcttcggggcgaaaactctcaaggatcttaccgctgttgagatccagttcgatgtaacccactcgtgcacccaactgatcttcagcatcttttactttcaccagcgtttctgggtgagcaaaaacaggaaggcaaaatgccgcaaaaaagggaataagggcgacacggaaatgttgaatactcatactcttcctttttcaat